European Patent Application EP 4 233 882 A1, published August 30, 2023. Title: MITOCHONDIRA COMPRISING ANTI-CANCER DRUG AND USE THEREOF. Applicant: Paean Biotechnology Inc. The sequence listing filed with the application follows.

SEQUENCE LISTING (102 sequences)

SEQ ID NO: 1 - DNA, 39 bp, Artificial Sequence
  T2p53 primer
aaaaaaccgcggtggtgaggagccgcagtcagatcctag

SEQ ID NO: 2 - DNA, 35 bp, Artificial Sequence
  Xp53 primer
aaaaaactcgagtgagtctgagtcaggcccttctg

SEQ ID NO: 3 - DNA, 1186 bp, Artificial Sequence
  nucleotides sequence coding p53
ccgcggtggtgaggagccgcagtcagatcctagcgtcgagccccctctgagtcaggaaacattttcagacctgtggaaactacttcctgaaaacaacgttctgtcccccttgccgtcccaagcaatggatgatttgatgctgtccccggacgatattgaacaatggttcactgaagacccaggtccagatgaagctcccagaatgccagaggctgctccccgcgtggcccctgcaccagcagctcctacaccggcggcccctgcaccagccccctcctggcccctgtcatcttctgtcccttcccagaaaacctaccagggcagctacggtttccgtctgggcttcttgcattctgggacagccaagtctgtgacttgcacgtactcccctgccctcaacaagatgttttgccaactggccaagacctgccctgtgcagctgtgggttgattccacacccccgcccggcacccgcgtccgcgccatggccatctacaagcagtcacagcacatgacggaggttgtgaggcgctgcccccaccatgagcgctgctcagatagcgatggtctggcccctcctcagcatcttatccgagtggaaggaaatttgcgtgtggagtatttggatgacagaaacacttttcgacatagtgtggtggtgccctatgagccgcctgaggttggctctgactgtaccaccatccactacaactacatgtgtaacagttcctgcatgggcggcatgaaccggaggcccatcctcaccatcatcacactggaagactccagtggtaatctactgggacggaacagctttgaggtgcgtgtttgtgcctgtcctgggagagaccggcgcacagaggaagagaatctccgcaagaaaggggagcctcaccacgagctgcccccagggagcactaagcgagcactgcccaacaacaccagctcctctccccagccaaagaagaaaccactggatggagaatatttcacccttcagatccgtgggcgtgagcgcttcgagatgttccgagagctgaatgaggccttggaactcaaggatgcccaggctgggaaggagccaggggggagcagggctcactccagccacctgaagtccaaaaagggtcagtctacctcccgccataaaaaactcatgttcaagacagaagggcctgactcagac

SEQ ID NO: 4 - DNA, 35 bp, Artificial Sequence
  NdeUB primer
ggattccatatgcaacttttcgtcaaaactctaac

SEQ ID NO: 5 - DNA, 27 bp, Artificial Sequence
  T2UB primer
atgaccaccgcggagtctcaacaccaa

SEQ ID NO: 6 - DNA, 1460 bp, Artificial Sequence
  nucleotides sequence coding UB-p53
atgggcagcagccatcatcatcatcatcacagcagcggcctggtgccgcgcggcagccatatgcaaatcttcgtcaaaactctaacagggaagactataaccctagaggttgaaccatccgacactattgaaaacgtcaaagctaaaattcaagataaagaaggtatccctccggatcagcagagattgatttttgctggtaagcaactagaagatggtagaaccttgtctgactacaacatccaaaaggaatctactcttcacttggtgttgagactccgcggtggtgaggagccgcagtcagatcctagcgtcgagccccctctgagtcaggaaacattttcagacctgtggaaactacttcctgaaaacaacgttctgtcccccttgccgtcccaagcaatggatgatttgatgctgtccccggacgatattgaacaatggttcactgaagacccaggtccagatgaagctcccagaatgccagaggctgctccccgcgtggcccctgcaccagcagctcctacaccggcggcccctgcaccagccccctcctggcccctgtcatcttctgtcccttcccagaaaacctaccagggcagctacggtttccgtctgggcttcttgcattctgggacagccaagtctgtgacttgcacgtactcccctgccctcaacaagatgttttgccaactggccaagacctgccctgtgcagctgtgggttgattccacacccccgcccggcacccgcgtccgcgccatggccatctacaagcagtcacagcacatgacggaggttgtgaggcgctgcccccaccatgagcgctgctcagatagcgatggtctggcccctcctcagcatcttatccgagtggaaggaaatttgcgtgtggagtatttggatgacagaaacacttttcgacatagtgtggtggtgccctatgagccgcctgaggttggctctgactgtaccaccatccactacaactacatgtgtaacagttcctgcatgggcggcatgaaccggaggcccatcctcaccatcatcacactggaagactccagtggtaatctactgggacggaacagctttgaggtgcgtgtttgtgcctgtcctgggagagaccggcgcacagaggaagagaatctccgcaagaaaggggagcctcaccacgagctgcccccagggagcactaagcgagcactgcccaacaacaccagctcctctccccagccaaagaagaaaccactggatggagaatatttcacccttcagatccgtgggcgtgagcgcttcgagatgttccgagagctgaatgaggccttggaactcaaggatgcccaggctgggaaggagccaggggggagcagggctcactccagccacctgaagtccaaaaagggtcagtctacctcccgccataaaaaactcatgttcaagacagaagggcctgatag

SEQ ID NO: 7 - DNA, 59 bp, Artificial Sequence
  NdeTOM70 primer
gaattccatatgaaaagttttataactcggaataaaactgcaattttcgcaactgttgc

SEQ ID NO: 8 - DNA, 38 bp, Artificial Sequence
  TOM70-AS primer
ggtgcatactactattatcaaacttttcgtcaaaactc

SEQ ID NO: 9 - DNA, 36 bp, Artificial Sequence
  TOM70UB-S primer
ggctacgtatttatttccaacttttcgtcaaaactc

SEQ ID NO: 10 - DNA, 24 bp, Artificial Sequence
  T2UB-AS primer
ggcaccaccgcggagtctcaacac

SEQ ID NO: 11 - DNA, 1515 bp, Artificial Sequence
  nucleotides sequence coding TOM70-UB-p53
atgaaaagttttataactcggaataaaactgcaattttcgcaactgttgctgctacgggaaccgctattggtgcatactactattatcaaatcttcgtcaaaactctaacagggaagactataaccctagaggttgaaccatccgacactattgaaaacgtcaaagctaaaattcaagataaagaaggtatccctccggatcagcagagattgatttttgctggtaagcaactagaagatggtagaaccttgtctgactacaacatccaaaaggaatctactcttcacttggtgttgagactccgcggtggtgaggagccgcagtcagatcctagcgtcgagccccctctgagtcaggaaacattttcagacctgtggaaactacttcctgaaaacaacgttctgtcccccttgccgtcccaagcaatggatgatttgatgctgtccccggacgatattgaacaatggttcactgaagacccaggtccagatgaagctcccagaatgccagaggctgctccccgcgtggcccctgcaccagcagctcctacaccggcggcccctgcaccagccccctcctggcccctgtcatcttctgtcccttcccagaaaacctaccagggcagctacggtttccgtctgggcttcttgcattctgggacagccaagtctgtgacttgcacgtactcccctgccctcaacaagatgttttgccaactggccaagacctgccctgtgcagctgtgggttgattccacacccccgcccggcacccgcgtccgcgccatggccatctacaagcagtcacagcacatgacggaggttgtgaggcgctgcccccaccatgagcgctgctcagatagcgatggtctggcccctcctcagcatcttatccgagtggaaggaaatttgcgtgtggagtatttggatgacagaaacacttttcgacatagtgtggtggtgccctatgagccgcctgaggttggctctgactgtaccaccatccactacaactacatgtgtaacagttcctgcatgggcggcatgaaccggaggcccatcctcaccatcatcacactggaagactccagtggtaatctactgggacggaacagctttgaggtgcgtgtttgtgcctgtcctgggagagaccggcgcacagaggaagagaatctccgcaagaaaggggagcctcaccacgagctgcccccagggagcactaagcgagcactgcccaacaacaccagctcctctccccagccaaagaagaaaccactggatggagaatatttcacccttcagatccgtgggcgtgagcgcttcgagatgttccgagagctgaatgaggccttggaactcaaggatgcccaggctgggaaggagccaggggggagcagggctcactccagccacctgaagtccaaaaagggtcagtctacctcccgccataaaaaactcatgttcaagacagaagggcctgactcagacctcgagcaccaccaccaccaccactag

SEQ ID NO: 12 - DNA, 59 bp, Artificial Sequence
  TOM70(G)3-AS primer
gcccccggatcctccacccccgcttccgccacctccataatagtagtatgcaccaatag

SEQ ID NO: 13 - DNA, 32 bp, Artificial Sequence
  (G)3UB-S primer
ggtggaggatccgggggcgcggaagccaaatc

SEQ ID NO: 14 - DNA, 32 bp, Artificial Sequence
  Xp53(noT) primer
aaaaaactcgaggtctgagtcaggcccttctg

SEQ ID NO: 15 - DNA, 1560 bp, Artificial Sequence
  nucleotides sequence coding TOM70-(GGGGS)3-UB-p53
atgaaaagttttataactcggaataaaactgcaattttcgcaactgttgctgctacgggaaccgctattggtgcatactactattatggaggtggcggaagcgggggtggaggatccgggggcggcggaagccaaatcttcgtcaaaactctaacagggaagactataaccctagaggttgaaccatccgacactattgaaaacgtcaaagctaaaattcaagataaagaaggtatccctccggatcagcagagattgatttttgctggtaagcaactagaagatggtagaaccttgtctgactacaacatccaaaaggaatctactcttcacttggtgttgagactccgcggtggtgaggagccgcagtcagatcctagcgtcgagccccctctgagtcaggaaacattttcagacctgtggaaactacttcctgaaaacaacgttctgtcccccttgccgtcccaagcaatggatgatttgatgctgtccccggacgatattgaacaatggttcactgaagacccaggtccagatgaagctcccagaatgccagaggctgctccccgcgtggcccctgcaccagcagctcctacaccggcggcccctgcaccagccccctcctggcccctgtcatcttctgtcccttcccagaaaacctaccagggcagctacggtttccgtctgggcttcttgcattctgggacagccaagtctgtgacttgcacgtactcccctgccctcaacaagatgttttgccaactggccaagacctgccctgtgcagctgtgggttgattccacacccccgcccggcacccgcgtccgcgccatggccatctacaagcagtcacagcacatgacggaggttgtgaggcgctgcccccaccatgagcgctgctcagatagcgatggtctggcccctcctcagcatcttatccgagtggaaggaaatttgcgtgtggagtatttggatgacagaaacacttttcgacatagtgtggtggtgccctatgagccgcctgaggttggctctgactgtaccaccatccactacaactacatgtgtaacagttcctgcatgggcggcatgaaccggaggcccatcctcaccatcatcacactggaagactccagtggtaatctactgggacggaacagctttgaggtgcgtgtttgtgcctgtcctgggagagaccggcgcacagaggaagagaatctccgcaagaaaggggagcctcaccacgagctgcccccagggagcactaagcgagcactgcccaacaacaccagctcctctccccagccaaagaagaaaccactggatggagaatatttcacccttcagatccgtgggcgtgagcgcttcgagatgttccgagagctgaatgaggccttggaactcaaggatgcccaggctgggaaggagccaggggggagcagggctcactccagccacctgaagtccaaaaagggtcagtctacctcccgccataaaaaactcatgttcaagacagaagggcctgactcagacctcgagcaccaccaccaccaccactag

SEQ ID NO: 16 - DNA, 51 bp, Artificial Sequence
  B(G)3p53
ggtggaggatccgggggcggcggaagcgaggagccgcagtcagatcctagc

SEQ ID NO: 17 - DNA, 1335 bp, Artificial Sequence
  nucleotides sequence coding TOM70-(GGGGS)3-p53
atgaaaagttttataactcggaataaaactgcaattttcgcaactgttgctgctacgggaaccgctattggtgcatactactattatggaggtggcggaagcgggggtggaggatccgggggcggcggaagcgaggagccgcagtcagatcctagcgtcgagccccctctgagtcaggaaacattttcagacctgtggaaactacttcctgaaaacaacgttctgtcccccttgccgtcccaagcaatggatgatttgatgctgtccccggacgatattgaacaatggttcactgaagacccaggtccagatgaagctcccagaatgccagaggctgctccccgcgtggcccctgcaccagcagctcctacaccggcggcccctgcaccagccccctcctggcccctgtcatcttctgtcccttcccagaaaacctaccagggcagctacggtttccgtctgggcttcttgcattctgggacagccaagtctgtgacttgcacgtactcccctgccctcaacaagatgttttgccaactggccaagacctgccctgtgcagctgtgggttgattccacacccccgcccggcacccgcgtccgcgccatggccatctacaagcagtcacagcacatgacggaggttgtgaggcgctgcccccaccatgagcgctgctcagatagcgatggtctggcccctcctcagcatcttatccgagtggaaggaaatttgcgtgtggagtatttggatgacagaaacacttttcgacatagtgtggtggtgccctatgagccgcctgaggttggctctgactgtaccaccatccactacaactacatgtgtaacagttcctgcatgggcggcatgaaccggaggcccatcctcaccatcatcacactggaagactccagtggtaatctactgggacggaacagctttgaggtgcgtgtttgtgcctgtcctgggagagaccggcgcacagaggaagagaatctccgcaagaaaggggagcctcaccacgagctgcccccagggagcactaagcgagcactgcccaacaacaccagctcctctccccagccaaagaagaaaccactggatggagaatatttcacccttcagatccgtgggcgtgagcgcttcgagatgttccgagagctgaatgaggccttggaactcaaggatgcccaggctgggaaggagccaggggggagcagggctcactccagccacctgaagtccaaaaagggtcagtctacctcccgccataaaaaactcatgttcaagacagaagggcctgactcagacctcgagcaccaccaccaccaccactag

SEQ ID NO: 18 - DNA, 32 bp, Artificial Sequence; identical to SEQ ID NO: 14
  Xp53(noT) primer

SEQ ID NO: 19 - DNA, 36 bp, Artificial Sequence
  XTOM7 primer
aaaaaactcgagtttgccattcgctggggctttatc

SEQ ID NO: 20 - DNA, 38 bp, Artificial Sequence
  LTOM7 primer
aaaaaagtcgacttatccccaaagtaggctcaaaacag

SEQ ID NO: 21 - DNA, 1578 bp, Artificial Sequence
  nucleotides sequence coding UB-p53-TOM7
atgggcagcagccatcatcatcatcatcacagcagcggcctggtgccgcgcggcagccatatgcaaatcttcgtcaaaactctaacagggaagactataaccctagaggttgaaccatccgacactattgaaaacgtcaaagctaaaattcaagataaagaaggtatccctccggatcagcagagattgatttttgctggtaagcaactagaagatggtagaaccttgtctgactacaacatccaaaaggaatctactcttcacttggtgttgagactccgcggtggtgaggagccgcagtcagatcctagcgtcgagccccctctgagtcaggaaacattttcagacctatggaaactacttcctgaaaacaacgttctgtcccccttgccgtcccaagcaatggatgatttgatgctgtccccggacgatattgaacaatggttcactgaagacccaggtccagatgaagctcccagaatgccagaggctgctccccgcgtggcccctgcaccagcagctcctacaccggcggcccctgcaccagccccctcctggcccctgtcatcttctgtcccttcccagaaaacctaccagggcagctacggtttccgtctgggcttcttgcattctgggacagccaagtctgtgacttgcacgtactcccctgccctcaacaagatgttttgccaactggccaagacctgccctgtgcagctgtgggttgattccacacccccgcccggcacccgcgtccgcgccatggccatctacaagcagtcacagcacatgacggaggttgtgaggcgctgcccccaccatgagcgctgctcagatagcgatggtctggcccctcctcagcatcttatccgagtggaaggaaatttgcgtgtggagtatttggatgacagaaacacttttcgacatagtgtggtggtgccctatgagccgcctgaggttggctctgactgtaccaccatccactacaactacatgtgtaacagttcctgcatgggcggcatgaaccggaggcccatcctcaccatcatcacactggaagactccagtggtaatctactgggacggaacagctttgaggtgcatgtttgtgcctgtcctgggagagaccggcgcacagaggaagagaatctccgcaagaaaggggagcctcaccacgagctgcccccagggagcactaagcgagcactgtccaacaacaccagctcctctccccagccaaagaagaaaccactggatggagaatatttcacccttcagatccgtgggcgtgagcgcttcgagatgttccgagagctgaatgaggccttggaactcaaggatgcccaggctgggaaggagccaggggggagcagggctcactccagccacctgaagtccaaaaagggtcagtctacctcccgccataaaaaactcatgttcaagacagaagggcctgactcagacctcgagtttgccattcgctggggctttatccctcttgtgatttacctgggatttaagaggggtgcagatcccggaatgcctgaaccaactgttttgagcctactttggggatag

SEQ ID NO: 22 - DNA, 35 bp, Artificial Sequence
  Rp53 primer
aaaaaagaattcatggtctgagtcaggcccttctg

SEQ ID NO: 23 - DNA, 1266 bp, Artificial Sequence
  nucleotides sequence coding p53-myc/His
atggaggagccgcagtcagatcctagcgtcgagccccctctgagtcaggaaacattttcagacctgtggaaactacttcctgaaaacaacgttctgtcccccttgccgtcccaagcaatggatgatttgatgctgtccccggacgatattgaacaatggttcactgaagacccaggtccagatgaagctcccagaatgccagaggctgctccccgcgtggcccctgcaccagcagctcctacaccggcggcccctgcaccagccccctcctggcccctgtcatcttctgtcccttcccagaaaacctaccagggcagctacggtttccgtctgggcttcttgcattctgggacagccaagtctgtgacttgcacgtactcccctgccctcaacaagatgttttgccaactggccaagacctgccctgtgcagctgtgggttgattccacacccccgcccggcacccgcgtccgcgccatggccatctacaagcagtcacagcacatgacggaggttgtgaggcgctgcccccaccatgagcgctgctcagatagcgatggtctggcccctcctcagcatcttatccgagtggaaggaaatttgcgtgtggagtatttggatgacagaaacacttttcgacatagtgtggtggtgccctatgagccgcctgaggttggctctgactgtaccaccatccactacaactacatgtgtaacagttcctgcatgggcggcatgaaccggaggcccatcctcaccatcatcacactggaagactccagtggtaatctactgggacggaacagctttgaggtgcgtgtttgtgcctgtcctgggagagaccggcgcacagaggaagagaatctccgcaagaaaggggagcctcaccacgagctgcccccagggagcactaagcgagcactgcccaacaacaccagctcctctccccagccaaagaagaaaccactggatggagaatatttcacccttcagatccgtgggcgtgagcgcttcgagatgttccgagagctgaatgaggccttggaactcaaggatgcccaggctgggaaggagccaggggggagcagggctcactccagccacctgaagtccaaaaagggtcagtctacctcccgccataaaaaactcatgttcaagacagaagggcctgactcagacctcgagtctagagggcccttcgaacaaaaactcatctcagaagaggatctgaatatgcataccggtcatcatcaccatcaccattga

SEQ ID NO: 24 - DNA, 51 bp, Artificial Sequence
  T2GZMB primer
aaaaaaccgcggtggtatcatcgggggacatgaggcacatgaggccaagcc

SEQ ID NO: 25 - DNA, 38 bp, Artificial Sequence
  XGZMB(noT) primer
aaaaaactcgaggtagcgtttcatggttttctttatcc

SEQ ID NO: 26 - DNA, 691 bp, Artificial Sequence
  nucleotides sequence coding GranzymeB
ccgcggtggtatcatcgggggacatgaggccaagccccactcccgcccctacatggcttatcttatgatctgggatcagaagtctctgaagaggtgcggtggcttcctgatacaagacgacttcgtgctgacagctgctcactgttggggaagctccataaatgtcaccttgggggcccacaatatcaaagaacaggagccgacccagcagtttatccctgtgaaaagacccatcccccatccagcctataatcctaagaacttctccaacgacatcatgctactgcagctggagagaaaggccaagcggaccagagctgtgcagcccctcaggctacctagcaacaaggcccaggtgaagccagggcagacatgcagtgtggccggctgggggcagacggcccccctgggaaaacactcacacacactacaagaggtgaagatgacagtgcaggaagatcgaaagtgcgaatctgacttacgccattattacgacagtaccattgagttgtgcgtgggggacccagagattaaaaagacttcctttaagggggactctggaggccctcttgtgtgtaacaaggtggcccagggcattgtctcctatggacgaaacaatggcatgcctccacgagcctgcaccaaagtctcaagctttgtacactggataaagaaaaccatgaaacgctac

SEQ ID NO: 27 - DNA, 1065 bp, Artificial Sequence
  nucleotides sequence coding TOM70-(GGGGS)3-UB-Granzyme B
atgaaaagttttataactcggaataaaactgcaattttcgcaactgttgctgctacgggaaccgctattggtgcatactactattatggaggtggcggaagcgggggtggaggatccgggggcggcggaagccaaatcttcgtcaaaactctaacagggaagactataaccctagaggttgaaccatccgacactattgaaaacgtcaaagctaaaattcaagataaagaaggtatccctccggatcagcagagattgatttttgctggtaagcaactagaagatggtagaaccttgtctgactacaacatccaaaaggaatctactcttcacttggtgttgagactccgcggtggtatcatcgggggacatgaggccaagccccactcccgcccctacatggcttatcttatgatctgggatcagaagtctctgaagaggtgcggtggcttcctgatacgagacgacttcgtgctgacagctgctcactgttggggaagctccataaatgtcaccttgggggcccacaatatcaaagaacaggagccgacccagcagtttatccctgtgaaaagacccatcccccatccagcctataatcctaagaacttctccaacgacatcatgctactgcagctggagagaaaggccaagcggaccagagctgtgcagcccctcaggctacctagcaacaaggcccaggtgaagccagggcagacatgcagtgtggccggctgggggcagacggcccccctgggaaaacactcacacacactacaagaggtgaagatgacagtgcaggaagatcgaaagtgcgaatctgacttacgccattattacgacagtaccattgagttgtgcgtgggggacccagagattaaaaagacttcctttaagggggactctggaggccctcttgtgtgtaacaaggtggcccagggcattgtctcctatggacgaaacaatggcatgcctccacgagcctgcaccaaagtctcaagctttgtacactggataaagaaaaccatgaaacgctacctcgagcaccaccaccaccaccactag

SEQ ID NO: 28 - DNA, 1083 bp, Artificial Sequence
  nucleotides sequence coding UB-Granzyme B-TOM7
atgggcagcagccatcatcatcatcatcacagcagcggcctggtgccgcgcggcagccatatgcaaatcttcgtcaaaactctaacagggaagactataaccctagaggttgaaccatccgacactattgaaaacgtcaaagctaaaattcaagataaagaaggtatccctccggatcagcagagattgatttttgctggtaagcaactagaagatggtagaaccttgtctgactacaacatccaaaaggaatctactcttcacttggtgttgagactccgcggtggtatcatcgggggacatgaggccaagccccactcccgcccctacatggcttatcttatgatctgggatcagaagtctctgaagaggtgcggtggcttcctgatacgagacgacttcgtgctgacagctgctcactgttggggaagctccataaatgtcaccttgggggcccacaatatcaaagaacaggagccgacccagcagtttatccctgtgaaaagacccatcccccatccagcctataatcctaagaacttctccaacgacatcatgctactgcagctggagagaaaggccaagcggaccagagctgtgcagcccctcaggctacctagcaacaaggcccaggtgaagccagggcagacatgcagtgtggccggctgggggcagacggcccccctgggaaaacactcacacacactacaagaggtgaagatgacagtgcaggaagatcgaaagtgcgaatctgacttacgccattattacgacagtaccattgagttgtgcgtgggggacccagagattaaaaagacttcctttaagggggactctggaggccctcttgtgtgtaacaaggtggcccagggcattgtctcctatggacgaaacaatggcatgcctccacgagcctgcaccaaagtctcaagctttgtacactggataaagaaaaccatgaaacgctacctcgagtttgccattcgctggggctttatccctcttgtgatttacctgggatttaagaggggtgcagatcccggaatgcctgaaccaactgttttgagcctactttggggatag

SEQ ID NO: 29 - DNA, 39 bp, Artificial Sequence
  T2RKIP primer
aaaaaaccgcggtggtccggtggacctcagcaagtggtc

SEQ ID NO: 30 - DNA, 41 bp, Artificial Sequence
  XRKIP(noT) primer
aaaaaactcgagcttcccagacagctgctcgtacagtttgg

SEQ ID NO: 31 - DNA, 568 bp, Artificial Sequence
  nucleotides sequence coding RKIP
ccgcggtggtccggtggacctcagcaagtggtccgggcccttgagcctgcaagaagtggacgagcagccgcagcacccactgcatgtcacctacgccggggcggcggtggacgagctgggcaaagtgctgacgcccacccaggttaagaatagacccaccagcatttcgtgggatggtcttgattcagggaagctctacaccttggtcctgacagacccggatgctcccagcaggaaggatcccaaatacagagaatggcatcatttcctggtggtcaacatgaagggcaatgacatcagcagtggcacagtcctctccgattatgtgggctcggggcctcccaagggcacaggcctccaccgctatgtctggctggtttacgagcaggacaggccgctaaagtgtgacgagcccatcctcagcaaccgatctggagaccaccgtggcaaattcaaggtggcgtccttccgtaaaaagtatgagctcagggccccggtggctggcacgtgttaccaggccgagtgggatgactatgtgcccaaactgtacgagcagctgtctgggaag

SEQ ID NO: 32 - DNA, 942 bp, Artificial Sequence
  nucleotides sequence coding TOM70-(GGGGS)3-UB-RKIP
atgaaaagttttataactcggaataaaactgcaattttcgcaactgttgctgctacgggaaccgctattggtgcatactactattatggaggtggcggaagcgggggtggaggatccgggggcggcggaagccaaatcttcgtcaaaactctaacagggaagactataaccctagaggttgaaccatccgacactattgaaaacgtcaaagctaaaattcaagataaagaaggtatccctccggatcagcagagattgatttttgctggtaagcaactagaagatggtagaaccttgtctgactacaacatccaaaaggaatctactcttcacttggtgttgagactccgcggtggtccggtggacctcagcaagtggtccgggcccttgagcctgcaagaagtggacgagcagccgcagcacccactgcatgtcacctacgccggggcggcggtggacgagctgggcaaagtgctgacgcccacccaggttaagaatagacccaccagcatttcgtgggatggtcttgattcagggaagctctacaccttggtcctgacagacccggatgctcccagcaggaaggatcccaaatacagagaatggcatcatttcctggtggtcaacatgaagggcaatgacatcagcagtggcacagtcctctccgattatgtgggctcggggcctcccaagggcacaggcctccaccgctatgtctggctggtttacgagcaggacaggccgctaaagtgtgacgagcccatcctcagcaaccgatctggagaccaccgtggcaaattcaaggtggcgtccttccgtaaaaagtatgagctcagggccccggtggctggcacgtgttaccaggccgagtgggatgactatgtgcccaaactgtacgagcagctgtctgggaagctcgagcaccaccaccaccaccactag

SEQ ID NO: 33 - DNA, 42 bp, Artificial Sequence
  T2PTEN primer
aaaaaaccgcggtggtacagccatcatcaaagagatcgttag

SEQ ID NO: 34 - DNA, 36 bp, Artificial Sequence
  XPTEN(noT) primer
aaaaaactcgaggacttttgtaatttgtgtatgctg

SEQ ID NO: 35 - DNA, 1216 bp, Artificial Sequence
  nucleotides sequence coding PTEN
ccgcggtggtacagccatcatcaaagagatcgttagcagaaacaaaaggagatatcaagaggatggattcgacttagacttgacctatatttatccaaacattattgctatgggatttcctgcagaaagacttgaaggcgtatacaggaacaatattgatgatgtagtaaggtttttggattcaaagcataaaaaccattacaagatatacaatctttgtgctgaaagacattatgacaccgccaaatttaattgcagagttgcacaatatccttttgaagaccataacccaccacagctagaacttatcaaacccttttgtgaagatcttgaccaatggctaagtgaagatgacaatcatgttgcagcaattcactgtaaagctggaaagggacgaactggtgtaatgatatgtgcatatttattacatcggggcaaatttttaaaggcacaagaggccctagatttctatggggaagtaaggaccagagacaaaaagggagtaactattcccagtcagaggcgctatgtgtattattatagctacctgttaaagaatcatctggattatagaccagtggcactgttgtttcacaagatgatgtttgaaactattccaatgttcagtggcggaacttgcaatcctcagtttgtggtctgccagctaaaggtgaagatatattcctccaattcaggacccacacgacgggaagacaagttcatgtactttgagttccctcagccgttacctgtgtgtggtgatatcaaagtagagttcttccacaaacagaacaagatgctaaaaaaggacaaaatgtttcacttttgggtaaatacattcttcataccaggaccagaggaaacctcagaaaaagtagaaaatggaagtctatgtgatcaagaaatcgatagcatttgcagtatagagcgtgcagataatgacaaggaatatctagtacttactttaacaaaaaatgatcttgacaaagcaaataaagacaaagccaaccgatacttttctccaaattttaaggtgaagctgtacttcacaaaaacagtagaggagccgtcaaatccagaggctagcagttcaacttctgtaacaccagatgttagtgacaatgaacctgatcattatagatattctgacaccactgactctgatccagagaatgaaccttttgatgaagatcagcatacacaaattacaaaagtc

SEQ ID NO: 36 - DNA, 1590 bp, Artificial Sequence
  nucleotides sequence coding TOM70-(GGGGS)3-UB-PTEN
atgaaaagttttataactcggaataaaactgcaattttcgcaactgttgctgctacgggaaccgctattggtgcatactactattatggaggtggcggaagcgggggtggaggatccgggggcggcggaagccaaatcttcgtcaaaactctaacagggaagactataaccctagaggttgaaccatccgacactattgaaaacgtcaaagctaaaattcaagataaagaaggtatccctccggatcagcagagattgatttttgctggtaagcaactagaagatggtagaaccttgtctgactacaacatccaaaaggaatctactcttcacttggtgttgagactccgcggtggtacagccatcatcaaagagatcgttagcagaaacaaaaggagatatcaagaggatggattcgacttagacttgacctatatttatccaaacattattgctatgggatttcctgcagaaagacttgaaggcgtatacaggaacaatattgatgatgtagtaaggtttttggattcaaagcataaaaaccattacaagatatacaatctttgtgctgaaagacattatgacaccgccaaatttaattgcagagttgcacaatatccttttgaagaccataacccaccacagctagaacttatcaaacccttttgtgaagatcttgaccaatggctaagtgaagatgacaatcatgttgcagcaattcactgtaaagctggaaagggacgaactggtgtaatgatatgtgcatatttattacatcggggcaaatttttaaaggcacaagaggccctagatttctatggggaagtaaggaccagagacaaaaagggagtaactattcccagtcagaggcgctatgtgtattattatagctacctgttaaagaatcatctggattatagaccagtggcactgttgtttcacaagatgatgtttgaaactattccaatgttcagtggcggaacttgcaatcctcagtttgtggtctgccagctaaaggtgaagatatattcctccaattcaggacccacacgacgggaagacaagttcatgtactttgagttccctcagccgttacctgtgtgtggtgatatcaaagtagagttcttccacaaacagaacaagatgctaaaaaaggacaaaatgtttcacttttgggtaaatacattcttcataccaggaccagaggaaacctcagaaaaagtagaaaatggaagtctatgtgatcaagaaatcgatagcatttgcagtatagagcgtgcagataatgacaaggaatatctagtacttactttaacaaaaaatgatcttgacaaagcaaataaagacaaagccaaccgatacttttctccaaattttaaggtgaagctgtacttcacaaaaacagtagaggagccgtcaaatccagaggctagcagttcaacttctgtaacaccagatgttagtgacaatgaacctgatcattatagatattctgacaccactgactctgatccagagaatgaaccttttgatgaagatcagcatacacaaattacaaaagtcctcgagcaccaccaccaccaccactag

SEQ ID NO: 37 - DNA, 739 bp, Artificial Sequence
  nucleotides sequence coding scFvHER2
ccgcggtggtgaagtgcaacttgttgagagtggcggaggactggtccaaccgggcggttcacttaggctctcatgtgcagcttcagggttcacgttcacggactatacaatggactgggtgaggcaagcccctggtaagggactggagtgggttgctgacgttaaccctaattccggtgggtccatctacaaccagcgattcaagggacgatttactctttcagtcgacagaagcaaaaacaccctctacctccagatgaactccttgcgggcagaggatacagcggtctactattgcgcgagaaacttgggaccaagcttctacttcgactactgggggcaaggaacgcttgttacggtttcaagcggaggtggaggaagtggaggtggcggttccggcggtggcggttcagatatacagatgacccaatcacccagttctcttagcgcgtctgtaggcgacagggtaaccataacctgcaaggcgtcccaggacgtgtcaattggagttgcctggtatcagcaaaaacctgggaaagctccgaagctcctgatttacagcgcatcttaccgatatactggtgtcccttcaaggttcagtggcagtggatctgggacagactttacgcttactatcagcagtctgcaacctgaggatttcgcgacctactactgtcagcagtattacatctatccgtacacgttcggtcaaggtacaaaggtagaaataaaacgcact

SEQ ID NO: 38 - DNA, 1125 bp, Artificial Sequence
  nucleotides sequence coding UB-scFvHER2-TOM7
atgggcagcagccatcatcatcatcatcacagcagcggcctggtgccgcgcggcagccatatgcaaatcttcgtcaaaactctaacagggaagactataaccctagaggttgaaccatccgacactattgaaaacgtcaaagctaaaattcaagataaagaaggtatccctccggatcagcagagattgatttttgctggtaagcaactagaagatggtagaaccttgtctgactacaacatccaaaaggaatctactcttcacttggtgttgagactccgcggtggtgaagtgcaacttgttgagagtggcggaggactggtccaaccgggcggttcacttaggctctcatgtgcagcttcagggttcacgttcacggactatacaatggactgggtgaggcaagcccctggtaagggactggagtgggttgctgacgttaaccctaattccggtgggtccatctacaaccagcgattcaagggacgatttactctttcagtcgacagaagcaaaaacaccctctacctccagatgaactccttgcgggcagaggatacagcggtctactattgcgcgagaaacttgggaccaagcttctacttcgactactgggggcaaggaacgcttgttacggtttcaagcggaggtggaggaagtggaggtggcggttccggcggtggcggttcagatatacagatgacccaatcacccagttctcttagcgcgtctgtaggcgacagggtaaccataacctgcaaggcgtcccaggacgtgtcaattggagttgcctggtatcagcaaaaacctgggaaagctccgaagctcctgatttacagcgcatcttaccgatatactggtgtcccttcaaggttcagtggcagtggatctgggacagactttacgcttactatcagcagtctgcaacctgaggatttcgcgacctactactgtcagcagtattacatctatccgtacacgttcggtcaaggtacaaaggtagaaataaaacgcacttttgccattcgctggggctttatccctcttgtgatttacctgggatttaagaggggtgcagatcccggaatgcctgaaccaactgttttgagcctactttggggatag

SEQ ID NO: 39 - DNA, 38 bp, Artificial Sequence
  RscFvHER2 primer
aaaaaagaattcatggaagtgcaacttgttgagagtgg

SEQ ID NO: 40 - DNA, 35 bp, Artificial Sequence
  XTOM7(noT) primer
aaaaaactcgagtccccaaagtaggctcaaaacag

SEQ ID NO: 41 - DNA, 924 bp, Artificial Sequence
  nucleotides sequence coding scFvHER2-TOM7-myc/His
atggaagtgcaacttgttgagagtggcggaggactggtccaaccgggcggttcacttaggctctcatgtgcagcttcagggttcacgttcacggactatacaatggactgggtgaggcaagcccctggtaagggactggagtgggttgctgacgttaaccctaattccggtgggtccatctacaaccagcgattcaagggacgatttactctttcagtcgacagaagcaaaaacaccctctacctccagatgaactccttgcgggcagaggatacagcggtctactattgcgcgagaaacttgggaccaagcttctacttcgactactgggggcaaggaacgcttgttacggtttcaagcggaggtggaggaagtggaggtggcggttccggcggtggcggttcagatatacagatgacccaatcacccagttctcttagcgcgtctgtaggcgacagggtaaccataacctgcaaggcgtcccaggacgtgtcaattggagttgcctggtatcagcaaaaacctgggaaagctccgaagctcctgatttacagcgcatcttaccgatatactggtgtcccttcaaggttcagtggcagtggatctgggacagactttacgcttactatcagcagtctgcaacctgaggatttcgcgacctactactgtcagcagtattacatctatccgtacacgttcggtcaaggtacaaaggtagaaataaaacgcacttttgccattcgctggggctttatccctcttgtgatttacctgggatttaagaggggtgcagatcccggaatgcctgaaccaactgttttgagcctactttggggactcgagtctagagggcccttcgaacaaaaactcatctcagaagaggatctgaatatgcataccggtcatcatcaccatcaccattga

SEQ ID NO: 42 - DNA, 760 bp, Artificial Sequence
  nucleotides sequence coding scFvMEL
ccgcggtggtacggacattgtgatgacccagtctcaaaaattcatgtccacatcagtaggagacagggtcagcgtcacctgcaaggccagtcagaatgtggatactaatgtagcctggtatcaacaaaaaccagggcaatctcctgaaccactgcttttctcggcatcctaccgttacactggagtccctgatcgcttcacaggcagtggatctgggacagatttcactctcaccatcagcaatgtgcagtctgaagacttggcagagtatttctgtcagcaatataacagctatcctctgacgttcggtggaggcaccaagctggagatcaaaggctccaccagcggcagcggtaagccaggctccggcgaaggcagcaccaaaggcgaagtgaaggttgaggagtctggaggaggcttggtgcaacctggaggatccatgaaactctcctgtgttgtctctggattcactttcggtaattactggatgaactgggtccgccagtctccagagaaggggcttgagtggattgcagaaattagattgaaatccaataattttgcaagatattatgcggagtctgtgaaagggaggttcaccatctcaagagatgattccaaaagtagtgtctacctgcaaatgatcaacctaagagctgaagatactggcatttattactgtaccagttatggtaactacgttgggcactattttgaccactggggccaaggcaccactctcaccgtctccctttgggga

SEQ ID NO: 43 - DNA, 1137 bp, Artificial Sequence
  nucleotides sequence coding UB-scFvMEL-TOM7
atgggcagcagccatcatcatcatcatcacagcagcggcctggtgccgcgcggcagccatatgcaaatcttcgtcaaaactctaacagggaagactataaccctagaggttgaaccatccgacactattgaaaacgtcaaagctaaaattcaagataaagaaggtatccctccggatcagcagagattgatttttgctggtaagcaactagaagatggtagaaccttgtctgactacaacatccaaaaggaatctactcttcacttggtgttgagactccgcggtggtacggacattgtgatgacccagtctcaaaaattcatgtccacatcagtaggagacagggtcagcgtcacctgcaaggccagtcagaatgtggatactaatgtagcctggtatcaacaaaaaccagggcaatctcctgaaccactgcttttctcggcatcctaccgttacactggagtccctgatcgcttcacaggcagtggatctgggacagatttcactctcaccatcagcaatgtgcagtctgaagacttggcagagtatttctgtcagcaatataacagctatcctctgacgttcggtggaggcaccaagctggagatcaaaggctccaccagcggcagcggtaagccaggctccggcgaaggcagcaccaaaggcgaagtgaaggttgaggagtctggaggaggcttggtgcaacctggaggatccatgaaactctcctgtgttgtctctggattcactttcggtaattactggatgaactgggtccgccagtctccagagaaggggcttgagtggattgcagaaattagattgaaatccaataattttgcaagatattatgcggagtctgtgaaagggaggttcaccatctcaagagatgattccaaaagtagtgtctacctgcaaatgatcaacctaagagctgaagatactggcatttattactgtaccagttatggtaactacgttgggcactattttgaccactggggccaaggcaccactctcaccgtctcctcatttgccattcgctggggctttatccctcttgtgatttacctgggatttaagaggggtgcagatcccggaatgcctgaaccaactgttttgagcctactttgggga

SEQ ID NO: 44 - DNA, 36 bp, Artificial Sequence
  RscFvMEL primer
aaaaaagaattcatgaaaacaagtaacccaggagtg

SEQ ID NO: 45 - DNA, 939 bp, Artificial Sequence
  nucleotides sequence coding scFvMEL-TOM7-myc/His
atgacggacattgtgatgacccagtctcaaaaattcatgtccacatcagtaggagacagggtcagcgtcacctgcaaggccagtcagaatgtggatactaatgtagcctggtatcaacaaaaaccagggcaatctcctgaaccactgcttttctcggcatcctaccgttacactggagtccctgatcgcttcacaggcagtggatctgggacagatttcactctcaccatcagcaatgtgcagtctgaagacttggcagagtatttctgtcagcaatataacagctatcctctgacgttcggtggaggcaccaagctggagatcaaaggctccaccagcggcagcggtaagccaggctccggcgaaggcagcaccaaaggcgaagtgaaggttgaggagtctggaggaggcttggtgcaacctggaggatccatgaaactctcctgtgttgtctctggattcactttcggtaattactggatgaactgggtccgccagtctccagagaaggggcttgagtggattgcagaaattagattgaaatccaataattttgcaagatattatgcggagtctgtgaaagggaggttcaccatctcaagagatgattccaaaagtagtgtctacctgcaaatgatcaacctaagagctgaagatactggcatttattactgtaccagttatggtaactacgttgggcactattttgaccactggggccaaggcaccactctcaccgtctcctcatttgccattcgctggggctttatccctcttgtgatttacctgggatttaagaggggtgcagatcccggaatgcctgaaccaactgttttgagcctactttggggactcgagtctagagggcccttcgaacaaaaactcatctcagaagaggatctgaatatgcataccggtcatcatcaccatcaccattga

SEQ ID NO: 46 - DNA, 750 bp, Artificial Sequence
  nucleotides sequence coding scFvPD-L1
atggacatcgtgatgagccagtctcccagcagcctggctgtgtctgctggggagaaggtgaccatgtcctgcaagagctcccagtccctgctgaacagccgcaccaggaagaactacctggcctggtaccagcagaagccaggccagagccccaagctcctcatctactgggccagcacccgggagagcggggtgcctgaccgcttcactggaagtggcagcggcacagacttcaccctgaccatcagctctgtgcaggccgaggacctggcagtgtactactgccagcaaagctatgatgtggtgacatttggagctggcaccaagctggagctgaagggaggtggcggaagcgggggtggaggatccgggggcggcggaagccaggtccaggtgcagcagagcggggctgagctggccgagcccggggcctctgtgaagatgagctgcaaggcttctggctacatcttcaccagctactggatgcactggctcaagcagaggcctgggcaggggctggagtggatcggctatatcaaccccagcagtgactacaatgaatattctgagaagttcatggacaaagccaccctgactgctgacaaggccagcaccaccgcctacatgcagctgatcagcctgacctcagaggacagcgctgtgtactactgtgcccggagcggctggctggtgcacggggactattattttgattattggggccagggcaccacactgacagtgagcagc

SEQ ID NO: 47 - DNA, 948 bp, Artificial Sequence
  nucleotides sequence coding scFvPD-L1-TOM7-myc/His
atggacatcgtgatgagccagtctcccagcagcctggctgtgtctgctggggagaaggtgaccatgtcctgcaagagctcccagtccctgctgaacagccgcaccaggaagaactacctggcctggtaccagcagaagccaggccagagccccaagctcctcatctactgggccagcacccgggagagcggggtgcctgaccgcttcactggaagtggcagcggcacagacttcaccctgaccatcagctctgtgcaggccgaggacctggcagtgtactactgccagcaaagctatgatgtggtgacatttggagctggcaccaagctggagctgaagggaggtggcggaagcgggggtggaggatccgggggcggcggaagccaggtccaggtgcagcagagcggggctgagctggccgagcccggggcctctgtgaagatgagctgcaaggcttctggctacatcttcaccagctactggatgcactggctcaagcagaggcctgggcaggggctggagtggatcggctatatcaaccccagcagtgactacaatgaatattctgagaagttcatggacaaagccaccctgactgctgacaaggccagcaccaccgcctacatgcagctgatcagcctgacctcagaggacagcgctgtgtactactgtgcccggagcggctggctggtgcacggggactattattttgattattggggccagggcaccacactgacagtgagcagcctcgagtttgccattcgctggggctttatccctcttgtgatttacctgggatttaagaggggtgcagatcccggaatgcctgaaccaactgttttgagcctactttggggactcgagtctagagggcccttcgaacaaaaactcatctcagaagaggatctgaatatgcataccggtcatcatcaccatcaccattga

SEQ ID NO: 48 - protein, 395 aa, Artificial Sequence
  amino acid sequence of p53
RGGEEPQSDPSVEPPLSQETFSDLWKLLPENNVLSPLPSQAMDDLMLSPDDIEQWFTEDPGPDEAPRMPEAAPRVAPAPAAPTPAAPAPAPSWPLSSSVPSQKTYQGSYGFRLGFLHSGTAKSVTCTYSPALNKMFCQLAKTCPVQLWVDSTPPPGTRVRAMAIYKQSQHMTEVVRRCPHHERCSDSDGLAPPQHLIRVEGNLRVEYLDDRNTFRHSVVVPYEPPEVGSDCTTIHYNYMCNSSCMGGMNRRPILTIITLEDSSGNLLGRNSFEVRVCACPGRDRRTEEENLRKKGEPHHELPPGSTKRALPNNTSSSPQPKKKPLDGEYFTLQIRGRERFEMFRELNEALELKDAQAGKEPGGSRAHSSHLKSKKGQSTSRHKKLMFKTEGPDSD

SEQ ID NO: 49 - protein, 488 aa, Artificial Sequence
  amino acid sequence of UB-p53
MGSSHHHHHHSSGLVPRGSHMQIFVKTLTGKTITLEVEPSDTIENVKAKIQDKEGIPPDQQRLIFAGKQLEDGRTLSDYNIQKESTLHLVLRLRGGEEPQSDPSVEPPLSQETFSDLWKLLPENNVLSPLPSQAMDDLMLSPDDIEQWFTEDPGPDEAPRMPEAAPRVAPAPAAPTPAAPAPAPSWPLSSSVPSQKTYQGSYGFRLGFLHSGTAKSVTCTYSPALNKMFCQLAKTCPVQLWVDSTPPPGTRVRAMAIYKQSQHMTEVVRRCPHHERCSDSDGLAPPQHLIRVEGNLRVEYLDDRNTFRHSVVVPYEPPEVGSDCTTIHYNYMCNSSCMGGMNRRPILTIITLEDSSGNLLGRNSFEVRVCACPGRDRRTEEENLRKKGEPHHELPPGSTKRALPNNTSSSPQPKKKPLDGEYFTLQIRGRERFEMFRELNEALELKDAQAGKEPGGSRAHSSHLKSKKGQSTSRHKKLMFKTEGPDSD

SEQ ID NO: 50 - protein, 504 aa, Artificial Sequence
  amino acid sequence of TOM70-UB-p53
MKSFITRNKTAIFATVAATGTAIGAYYYYQIFVKTLTGKTITLEVEPSDTIENVKAKIQDKEGIPPDQQRLIFAGKQLEDGRTLSDYNIQKESTLHLVLRLRGGEEPQSDPSVEPPLSQETFSDLWKLLPENNVLSPLPSQAMDDLMLSPDDIEQWFTEDPGPDEAPRMPEAAPRVAPAPAAPTPAAPAPAPSWPLSSSVPSQKTYQGSYGFRLGFLHSGTAKSVTCTYSPALNKMFCQLAKTCPVQLWVDSTPPPGTRVRAMAIYKQSQHMTEVVRRCPHHERCSDSDGLAPPQHLIRVEGNLRVEYLDDRNTFRHSVVVPYEPPEVGSDCTTIHYNYMCNSSCMGGMNRRPILTIITLEDSSGNLLGRNSFEVRVCACPGRDRRTEEENLRKKGEPHHELPPGSTKRALPNNTSSSPQPKKKPLDGEYFTLQIRGRERFEMFRELNEALELKDAQAGKEPGGSRAHSSHLKSKKGQSTSRHKKLMFKTEGPDSDLEHHHHHH

SEQ ID NO: 51 - protein, 519 aa, Artificial Sequence
  amino acid sequence of TOM70-(GGGGS)3-UB-p53
MKSFITRNKTAIFATVAATGTAIGAYYYYGGGGSGGGGSGGGGSQIFVKTLTGKTITLEVEPSDTIENVKAKIQDKEGIPPDQQRLIFAGKQLEDGRTLSDYNIQKESTLHLVLRLRGGEEPQSDPSVEPPLSQETFSDLWKLLPENNVLSPLPSQAMDDLMLSPDDIEQWFTEDPGPDEAPRMPEAAPRVAPAPAAPTPAAPAPAPSWPLSSSVPSQKTYQGSYGFRLGFLHSGTAKSVTCTYSPALNKMFCQLAKTCPVQLWVDSTPPPGTRVRAMAIYKQSQHMTEVVRRCPHHERCSDSDGLAPPQHLIRVEGNLRVEYLDDRNTFRHSVVVPYEPPEVGSDCTTIHYNYMCNSSCMGGMNRRPILTIITLEDSSGNLLGRNSFEVRVCACPGRDRRTEEENLRKKGEPHHELPPGSTKRALPNNTSSSPQPKKKPLDGEYFTLQIRGRERFEMFRELNEALELKDAQAGKEPGGSRAHSSHLKSKKGQSTSRHKKLMFKTEGPDSDLEHHHHHH

SEQ ID NO: 52 - protein, 444 aa, Artificial Sequence
  amino acid sequence of TOM70-(GGGGS)3-p53
MKSFITRNKTAIFATVAATGTAIGAYYYYGGGGSGGGGSGGGGSEEPQSDPSVEPPLSQETFSDLWKLLPENNVLSPLPSQAMDDLMLSPDDIEQWFTEDPGPDEAPRMPEAAPRVAPAPAAPTPAAPAPAPSWPLSSSVPSQKTYQGSYGFRLGFLHSGTAKSVTCTYSPALNKMFCQLAKTCPVQLWVDSTPPPGTRVRAMAIYKQSQHMTEVVRRCPHHERCSDSDGLAPPQHLIRVEGNLRVEYLDDRNTFRHSVVVPYEPPEVGSDCTTIHYNYMCNSSCMGGMNRRPILTIITLEDSSGNLLGRNSFEVRVCACPGRDRRTEEENLRKKGEPHHELPPGSTKRALPNNTSSSPQPKKKPLDGEYFTLQIRGRERFEMFRELNEALELKDAQAGKEPGGSRAHSSHLKSKKGQSTSRHKKLMFKTEGPDSDLEHHHHHH

SEQ ID NO: 53 - protein, 525 aa, Artificial Sequence
  amino acid sequence of UB-p53-TOM7
MGSSHHHHHHSSGLVPRGSHMQIFVKTLTGKTITLEVEPSDTIENVKAKIQDKEGIPPDQQRLIFAGKQLEDGRTLSDYNIQKESTLHLVLRLRGGEEPQSDPSVEPPLSQETFSDLWKLLPENNVLSPLPSQAMDDLMLSPDDIEQWFTEDPGPDEAPRMPEAAPRVAPAPAAPTPAAPAPAPSWPLSSSVPSQKTYQGSYGFRLGFLHSGTAKSVTCTYSPALNKMFCQLAKTCPVQLWVDSTPPPGTRVRAMAIYKQSQHMTEVVRRCPHHERCSDSDGLAPPQHLIRVEGNLRVEYLDDRNTFRHSVVVPYEPPEVGSDCTTIHYNYMCNSSCMGGMNRRPILTIITLEDSSGNLLGRNSFEVHVCACPGRDRRTEEENLRKKGEPHHELPPGSTKRALSNNTSSSPQPKKKPLDGEYFTLQIRGRERFEMFRELNEALELKDAQAGKEPGGSRAHSSHLKSKKGQSTSRHKKLMFKTEGPDSDLEFAIRWGFIPLVIYLGFKRGADPGMPEPTVLSLLWG

SEQ ID NO: 54 - protein, 421 aa, Artificial Sequence
  amino acid sequence of p53-myc/His
MEEPQSDPSVEPPLSQETFSDLWKLLPENNVLSPLPSQAMDDLMLSPDDIEQWFTEDPGPDEAPRMPEAAPRVAPAPAAPTPAAPAPAPSWPLSSSVPSQKTYQGSYGFRLGFLHSGTAKSVTCTYSPALNKMFCQLAKTCPVQLWVDSTPPPGTRVRAMAIYKQSQHMTEVVRRCPHHERCSDSDGLAPPQHLIRVEGNLRVEYLDDRNTFRHSVVVPYEPPEVGSDCTTIHYNYMCNSSCMGGMNRRPILTIITLEDSSGNLLGRNSFEVRVCACPGRDRRTEEENLRKKGEPHHELPPGSTKRALPNNTSSSPQPKKKPLDGEYFTLQIRGRERFEMFRELNEALELKDAQAGKEPGGSRAHSSHLKSKKGQSTSRHKKLMFKTEGPDSDLESRGPFEQKLISEEDLNMHTGHHHHHH

SEQ ID NO: 55 - protein, 230 aa, Artificial Sequence
  amino acid sequence of GranzymeB
RGGIIGGHEAKPHSRPYMAYLMIWDQKSLKRCGGFLIQDDFVLTAAHCWGSSINVTLGAHNIKEQEPTQQFIPVKRPIPHPAYNPKNFSNDIMLLQLERKAKRTRAVQPLRLPSNKAQVKPGQTCSVAGWGQTAPLGKHSHTLQEVKMTVQEDRKCESDLRHYYDSTIELCVGDPEIKKTSFKGDSGGPLVCNKVAQGIVSYGRNNGMPPRACTKVSSFVHWIKKTMKRY

SEQ ID NO: 56 - protein, 354 aa, Artificial Sequence
  amino acid sequence of TOM70-(GGGGS)3-UB-Granzyme B
MKSFITRNKTAIFATVAATGTAIGAYYYYGGGGSGGGGSGGGGSQIFVKTLTGKTITLEVEPSDTIENVKAKIQDKEGIPPDQQRLIFAGKQLEDGRTLSDYNIQKESTLHLVLRLRGGIIGGHEAKPHSRPYMAYLMIWDQKSLKRCGGFLIRDDFVLTAAHCWGSSINVTLGAHNIKEQEPTQQFIPVKRPIPHPAYNPKNFSNDIMLLQLERKAKRTRAVQPLRLPSNKAQVKPGQTCSVAGWGQTAPLGKHSHTLQEVKMTVQEDRKCESDLRHYYDSTIELCVGDPEIKKTSFKGDSGGPLVCNKVAQGIVSYGRNNGMPPRACTKVSSFVHWIKKTMKRYLEHHHHHH

SEQ ID NO: 57 - protein, 360 aa, Artificial Sequence
  amino acid sequence of UB-Granzyme B-TOM7
MGSSHHHHHHSSGLVPRGSHMQIFVKTLTGKTITLEVEPSDTIENVKAKIQDKEGIPPDQQRLIFAGKQLEDGRTLSDYNIQKESTLHLVLRLRGGIIGGHEAKPHSRPYMAYLMIWDQKSLKRCGGFLIRDDFVLTAAHCWGSSINVTLGAHNIKEQEPTQQFIPVKRPIPHPAYNPKNFSNDIMLLQLERKAKRTRAVQPLRLPSNKAQVKPGQTCSVAGWGQTAPLGKHSHTLQEVKMTVQEDRKCESDLRHYYDSTIELCVGDPEIKKTSFKGDSGGPLVCNKVAQGIVSYGRNNGMPPRACTKVSSFVHWIKKTMKRYLEFAIRWGFIPLVIYLGFKRGADPGMPEPTVLSLLWG

SEQ ID NO: 58 - protein, 189 aa, Artificial Sequence
  amino acid sequence of RKIP
RGGPVDLSKWSGPLSLQEVDEQPQHPLHVTYAGAAVDELGKVLTPTQVKNRPTSISWDGLDSGKLYTLVLTDPDAPSRKDPKYREWHHFLVVNMKGNDISSGTVLSDYVGSGPPKGTGLHRYVWLVYEQDRPLKCDEPILSNRSGDHRGKFKVASFRKKYELRAPVAGTCYQAEWDDYVPKLYEQLSGK

SEQ ID NO: 59 - protein, 313 aa, Artificial Sequence
  amino acid sequence of TOM70-(GGGGS)3-UB-RKIP
MKSFITRNKTAIFATVAATGTAIGAYYYYGGGGSGGGGSGGGGSQIFVKTLTGKTITLEVEPSDTIENVKAKIQDKEGIPPDQQRLIFAGKQLEDGRTLSDYNIQKESTLHLVLRLRGGPVDLSKWSGPLSLQEVDEQPQHPLHVTYAGAAVDELGKVLTPTQVKNRPTSISWDGLDSGKLYTLVLTDPDAPSRKDPKYREWHHFLVVNMKGNDISSGTVLSDYVGSGPPKGTGLHRYVWLVYEQDRPLKCDEPILSNRSGDHRGKFKVASFRKKYELRAPVAGTCYQAEWDDYVPKLYEQLSGKLEHHHHHH

SEQ ID NO: 60 - protein, 405 aa, Artificial Sequence
  amino acid sequence of PTEN
RGGTAIIKEIVSRNKRRYQEDGFDLDLTYIYPNIIAMGFPAERLEGVYRNNIDDVVRFLDSKHKNHYKIYNLCAERHYDTAKFNCRVAQYPFEDHNPPQLELIKPFCEDLDQWLSEDDNHVAAIHCKAGKGRTGVMICAYLLHRGKFLKAQEALDFYGEVRTRDKKGVTIPSQRRYVYYYSYLLKNHLDYRPVALLFHKMMFETIPMFSGGTCNPQFVVCQLKVKIYSSNSGPTRREDKFMYFEFPQPLPVCGDIKVEFFHKQNKMLKKDKMFHFWVNTFFIPGPEETSEKVENGSLCDQEIDSICSIERADNDKEYLVLTLTKNDLDKANKDKANRYFSPNFKVKLYFTKTVEEPSNPEASSSTSVTPDVSDNEPDHYRYSDTTDSDPENEPFDEDQHTQITKV

SEQ ID NO: 61 - protein, 529 aa, Artificial Sequence
  amino acid sequence of TOM70-(GGGGS)3-UB-PTEN
MKSFITRNKTAIFATVAATGTAIGAYYYYGGGGSGGGGSGGGGSQIFVKTLTGKTITLEVEPSDTIENVKAKIQDKEGIPPDQQRLIFAGKQLEDGRTLSDYNIQKESTLHLVLRLRGGTAIIKEIVSRNKRRYQEDGFDLDLTYIYPNIIAMGFPAERLEGVYRNNIDDVVRFLDSKHKNHYKIYNLCAERHYDTAKFNCRVAQYPFEDHNPPQLELIKPFCEDLDQWLSEDDNHVAAIHCKAGKGRTGVMICAYLLHRGKFLKAQEALDFYGEVRTRDKKGVTIPSQRRYVYYYSYLLKNHLDYRPVALLFHKMMFETIPMFSGGTCNPQFVVCQLKVKIYSSNSGPTRREDKFMYFEFPQPLPVCGDIKVEFFHKQNKMLKKDKMFHFWVNTFFIPGPEETSEKVENGSLCDQEIDSICSIERADNDKEYLVLTLTKNDLDKANKDKANRYFSPNFKVKLYFTKTVEEPSNPEASSSTSVTPDVSDNEPDHYRYSDTTDSDPENEPFDEDQHTQITKVLEHHHHHH

SEQ ID NO: 62 - protein, 246 aa, Artificial Sequence
  amino acid sequence of scFvHER2
RGGEVQLVESGGGLVQPGGSLRLSCAASGFTFTDYTMDWVRQAPGKGLEWVADVNPNSGGSIYNQRFKGRFTLSVDRSKNTLYLQMNSLRAEDTAVYYCARNLGPSFYFDYWGQGTLVTVSSGGGGSGGGGSGGGGSDIQMTQSPSSLSASVGDRVTITCKASQDVSIGVAWYQQKPGKAPKLLIYSASYRYTGVPSRFSGSGSGTDFTLTISSLQPEDFATYYCQQYYIYPYTFGQGTKVEIKRT

SEQ ID NO: 63 - protein, 374 aa, Artificial Sequence
  amino acid sequence of UB-scFvHER2-TOM7
MGSSHHHHHHSSGLVPRGSHMQIFVKTLTGKTITLEVEPSDTIENVKAKIQDKEGIPPDQQRLIFAGKQLEDGRTLSDYNIQKESTLHLVLRLRGGEVQLVESGGGLVQPGGSLRLSCAASGFTFTDYTMDWVRQAPGKGLEWVADVNPNSGGSIYNQRFKGRFTLSVDRSKNTLYLQMNSLRAEDTAVYYCARNLGPSFYFDYWGQGTLVTVSSGGGGSGGGGSGGGGSDIQMTQSPSSLSASVGDRVTITCKASQDVSIGVAWYQQKPGKAPKLLIYSASYRYTGVPSRFSGSGSGTDFTLTISSLQPEDFATYYCQQYYIYPYTFGQGTKVEIKRTFAIRWGFIPLVIYLGFKRGADPGMPEPTVLSLLWG

SEQ ID NO: 64 - protein, 307 aa, Artificial Sequence
  amino acid sequence of scFvHER2-TOM7-myc/His
MEVQLVESGGGLVQPGGSLRLSCAASGFTFTDYTMDWVRQAPGKGLEWVADVNPNSGGSIYNQRFKGRFTLSVDRSKNTLYLQMNSLRAEDTAVYYCARNLGPSFYFDYWGQGTLVTVSSGGGGSGGGGSGGGGSDIQMTQSPSSLSASVGDRVTITCKASQDVSIGVAWYQQKPGKAPKLLIYSASYRYTGVPSRFSGSGSGTDFTLTISSLQPEDFATYYCQQYYIYPYTFGQGTKVEIKRTFAIRWGFIPLVIYLGFKRGADPGMPEPTVLSLLWGLESRGPFEQKLISEEDLNMHTGHHHHHH

SEQ ID NO: 65 - protein, 251 aa, Artificial Sequence
  amino acid sequence of scFvMEL
RGGTDIVMTQSQKFMSTSVGDRVSVTCKASQNVDTNVAWYQQKPGQSPEPLLFSASYRYTGVPDRFTGSGSGTDFTLTISNVQSEDLAEYFCQQYNSYPLTFGGGTKLEIKGSTSGSGKPGSGEGSTKGEVKVEESGGGLVQPGGSMKLSCVVSGFTFGNYWMNWVRQSPEKGLEWIAEIRLKSNNFARYYAESVKGRFTISRDDSKSSVYLQMINLRAEDTGIYYCTSYGNYVGHYFDHWGQGTTLTVSS

SEQ ID NO: 66 - protein, 378 aa, Artificial Sequence
  amino acid sequence of UB-scFvMEL-TOM7
MGSSHHHHHHSSGLVPRGSHMQIFVKTLTGKTITLEVEPSDTIENVKAKIQDKEGIPPDQQRLIFAGKQLEDGRTLSDYNIQKESTLHLVLRLRGGTDIMTQSQKFMSTSVGDRVSVTCKASQNVDTNVAWYQQKPGQSPEPLLFSASYRYTGVPDRFTGSGSGTDFTLTISNVQSEDLAEYFCQQYNSYPLTFGGGTKLEIKGSTSGSGKPGSGEGSTKGEVKVEESGGGLVQPGGSMKLSCVVSGFTFGNYWMNWVRQSPEKGLEWIAEIRLKSNNFARYYAESVKGRFTISRDDSKSSVYLQMINLRAEDTGIYYCTSYGNYVGHYFDHWGQGTTLTVSSFAIRWGFIPLVIYLGFKRGADPGMPEPTVLSLLWG

SEQ ID NO: 67 - protein, 312 aa, Artificial Sequence
  amino acid sequence of scFvMEL-TOM7-myc/His
MTDIVMTQSQKFMSTSVGDRVSVTCKASQNVDTNVAWYQQKPGQSPEPLLFSASYRYTGVPDRFTGSGSGTDFTLTISNVQSEDLAEYFCQQYNSYPLTFGGGTKLEIKGSTSGSGKPGSGEGSTKGEVKVEESGGGLVQPGGSMKLSCVVSGFTFGNYWMNWVRQSPEKGLEWIAEIRLKSNNFARYYAESVKGRFTISRDDSKSSVYLQMINLRAEDTGIYYCTSYGNYVGHYFDHWGQGTTLTVSSFAIRWGFIPLVIYLGFKRGADPGMPEPTVLSLLWGLESRGPFEQKLISEEDLNMHTGHHHHHH

SEQ ID NO: 68 - protein, 250 aa, Artificial Sequence
  amino acid sequence of scFvPD-L1
MDIVMSQSPSSLAVSAGEKVTMSCKSSQSLLNSRTRKNYLAWYQQKPGQSPKLLIYWASTRESGVPDRFTGSGSGTDFTLTISSVQAEDLAVYYCQQSYDVVTFGAGTKLELKGGGGSGGGGSGGGGSQVQVQQSGAELAEPGASVKMSCKASGYIFTSYWMHWLKQRPGQGLEWIGYINPSSDYNEYSEKFMDKATLTADKASTTAYMQLISLTSEDSAVYYCARSGWLVHGDYYFDYWGQGTTLTVSS

SEQ ID NO: 69 - protein, 315 aa, Artificial Sequence
  amino acid sequence of scFvPD-L1-TOM7-myc/His
MDIVMSQSPSSLAVSAGEKVTMSCKSSQSLLNSRTRKNYLAWYQQKPGQSPKLLIYWASTRESGVPDRFTGSGSGTDFTLTISSVQAEDLAVYYCQQSYDVVTFGAGTKLELKGGGGSGGGGSGGGGSQVQVQQSGAELAEPGASVKMSCKASGYIFTSYWMHWLKQRPGQGLEWIGYINPSSDYNEYSEKFMDKATLTADKASTTAYMQLISLTSEDSAVYYCARSGWLVHGDYYFDYWGQGTTLTVSSLEFAIRWGFIPLVIYLGFKRGADPGMPEPTVLSLLWGLESRGPFEQKLISEEDLNMHTGHHHHHH

SEQ ID NO: 70 - DNA, 15 bp, Artificial Sequence
  linker
ggggsggggsggggs

SEQ ID NO: 71 - protein, 75 aa, Artificial Sequence
  amino acid sequence of ubiquitin
QLFVKTLTGKTVTLEVESSDTIDNVKSKIQDKEGIPPDQQRLIFAGKQLEDGRTLSDYNIQKESTLHLVLRLRGG

SEQ ID NO: 72 - DNA, 225 bp, Artificial Sequence
  nucleotides sequence coding ubiquitin
caacttttcgtcaaaactctaacagggaagactgtaaccctagaggttgaatcttccgacactattgacaacgtcaaaagtaaaattcaagataaagaaggtatccctccggatcagcagagattgatttttgctggtaagcaactagaagatggtagaaccttgtctgactacaacatccaaaaggaatctactcttcacttggtgttgagactccgcggtggt

SEQ ID NO: 73 - protein, 400 aa, Artificial Sequence
  amino acid sequence of p53
EEPQSDPSVEPPLSQETFSDLWKLLPENNVLSPLPSQAMDDLMLSPDDIEQWFTEDPGPDEAPRMPEAAPRVAPAPAAPTPAAPAPAPSWPLSSSVPSQKTYQGSYGFRLGFLHSGTAKSVTCTYSPALNKMFCQLAKTCPVQLWVDSTPPPGTRVRAMAIYKQSQHMTEVVRRCPHHERCSDSDGLAPPQHLIRVEGNLRVEYLDDRNTFRHSVVVPYEPPEVGSDCTTIHYNYMCNSSCMGGMNRRPILTIITLEDSSGNLLGRNSFEVRVCACPGRDRRTEEENLRKKGEPHHELPPGSTKRALPNNTSSSPQPKKKPLDGEYFTLQIRGRERFEMFRELNEALELKDAQAGKEPGGSRAHSSHLKSKKGQSTSRHKKLMFKTEGPDSDLEHHHHHH

SEQ ID NO: 74 - DNA, 1203 bp, Artificial Sequence
  nucleotides sequence coding p53
gaggagccgcagtcagatcctagcgtcgagccccctctgagtcaggaaacattttcagacctgtggaaactacttcctgaaaacaacgttctgtcccccttgccgtcccaagcaatggatgatttgatgctgtccccggacgatattgaacaatggttcactgaagacccaggtccagatgaagctcccagaatgccagaggctgctccccgcgtggcccctgcaccagcagctcctacaccggcggcccctgcaccagccccctcctggcccctgtcatcttctgtcccttcccagaaaacctaccagggcagctacggtttccgtctgggcttcttgcattctgggacagccaagtctgtgacttgcacgtactcccctgccctcaacaagatgttttgccaactggccaagacctgccctgtgcagctgtgggttgattccacacccccgcccggcacccgcgtccgcgccatggccatctacaagcagtcacagcacatgacggaggttgtgaggcgctgcccccaccatgagcgctgctcagatagcgatggtctggcccctcctcagcatcttatccgagtggaaggaaatttgcgtgtggagtatttggatgacagaaacacttttcgacatagtgtggtggtgccctatgagccgcctgaggttggctctgactgtaccaccatccactacaactacatgtgtaacagttcctgcatgggcggcatgaaccggaggcccatcctcaccatcatcacactggaagactccagtggtaatctactgggacggaacagctttgaggtgcgtgtttgtgcctgtcctgggagagaccggcgcacagaggaagagaatctccgcaagaaaggggagcctcaccacgagctgcccccagggagcactaagcgagcactgcccaacaacaccagctcctctccccagccaaagaagaaaccactggatggagaatatttcacccttcagatccgtgggcgtgagcgcttcgagatgttccgagagctgaatgaggccttggaactcaaggatgcccaggctgggaaggagccaggggggagcagggctcactccagccacctgaagtccaaaaagggtcagtctacctcccgccataaaaaactcatgttcaagacagaagggcctgactcagacctcgagcaccaccaccaccaccactag

SEQ ID NO: 75 - protein, 29 aa, Artificial Sequence
  TOM70 of S. cerevisiae
MKSFITRNKTAIFATVAATGTAIGAYYYY

SEQ ID NO: 76 - protein, 60 aa, Artificial Sequence
  TOM70 of Homo sapiens
MAASKPVEAAVVAAAVPSSGSGVGGGGTAGPGTGGLPRWQLALAVGAPLLLGAGAIYLWS

SEQ ID NO: 77 - protein, 29 aa, Artificial Sequence
  TOM20 of S. cerevisiae
MSQSNPILRGLAITTAIAALSATGYAIYF

SEQ ID NO: 78 - protein, 24 aa, Artificial Sequence
  TOM20 of Homo sapiens
MVGRNSAIAAGVCGALFIGYCIYF

SEQ ID NO: 79 - protein, 22 aa, Artificial Sequence
  OM45 of S. cerevisiae
MSSRIIVGSAALAAAITASIMV

SEQ ID NO: 80 - protein, 23 aa, Artificial Sequence
  TOM5 of S. cerevisiae
AAYVAAFLWVSPMIWHLVKKQWK

SEQ ID NO: 81 - protein, 24 aa, Artificial Sequence
  TOM5 of Homo sapiens
IRNFLIYVALLRVTPFILKKLDSI

SEQ ID NO: 82 - protein, 41 aa, Artificial Sequence
  TOM7 of S. cerevisiae
ILTLTHNVAHYGWIPFVLYLGWAHTSNRPNFLNLLSPLPSV

SEQ ID NO: 83 - protein, 35 aa, Artificial Sequence
  TOM7 of Homo sapiens
FAIRWGFIPLVIYLGFKRGADPGMPEPTVLSLLWG

SEQ ID NO: 84 - protein, 55 aa, Artificial Sequence
  TOM22 of S. cerevisiae
LAWTLTTTALLLGVPLSLSILAEQQLIEMEKTFDLQSDANNILAQGEKDAAATAN

SEQ ID NO: 85 - protein, 60 aa, Artificial Sequence
  TOM22 of Homo sapiens
AALWIGTTSFMILVLPVVFETEKLQMEQQQQLQQRQILLGPNTGLSGGMPGALPSLPGKI

SEQ ID NO: 86 - protein, 25 aa, Artificial Sequence
  Fis1 of S. cerevisiae
GVVVAGGVLAGAVAVASFFLRNKRR

SEQ ID NO: 87 - protein, 31 aa, Artificial Sequence
  Fis1 of Homo sapiens
GLVGMAIVGGMALGVAGLAGLIGLAVSKSKS

SEQ ID NO: 88 - protein, 25 aa, Artificial Sequence
  Bcl-2 alpha of Homo sapiens
LSLKTLLSLALVGACITLGAYLGHK

SEQ ID NO: 89 - protein, 19 aa, Artificial Sequence
  VAMP1 of S. cerevisiae
MIMLGAICAIIVVVIVRRD

SEQ ID NO: 90 - protein, 22 aa, Artificial Sequence
  VAMP1 of Homo sapiens
MMIMLGAICAIIVVVIVIYFFT

SEQ ID NO: 91 - DNA, 60 bp, Artificial Sequence
  P53-promter-S
gggcatgctcgggcatgcccgggcatgctcgggcatgcccgggcatgctcgggcatgccc

SEQ ID NO: 92 - DNA, 60 bp, Artificial Sequence
  P53-promter-AS
gggcatgcccgagcatgcccgggcatgcccgagcatgcccgggcatgcccgagcatgccc

SEQ ID NO: 93 - DNA, 945 bp, Artificial Sequence
  nucleotides sequence coding scFvPDL1-myc-TOM7
atggacatcgtgatgagccagtctcccagcagcctggctgtgtctgctggggagaaggtgaccatgtcctgcaagagctcccagtccctgctgaacagccgcaccaggaagaactacctggcctggtaccagcagaagccaggccagagccccaagctcctcatctactgggccagcacccgggagagcggggtgcctgaccgcttcactggaagtggcagcggcacagacttcaccctgaccatcagctctgtgcaggccgaggacctggcagtgtactactgccagcaaagctatgatgtggtgacatttggagctggcaccaagctggagctgaagggaggtggcggaagcgggggtggaggatccgggggcggcggaagccaggtccaggtgcagcagagcggggctgagctggccgagcccggggcctctgtgaagatgagctgcaaggcttctggctacatcttcaccagctactggatgcactggctcaagcagaggcctgggcaggggctggagtggatcggctatatcaaccccagcagtgactacaatgaatattctgagaagttcatggacaaagccaccctgactgctgacaaggccagcaccaccgcctacatgcagctgatcagcctgacctcagaggacagcgctgtgtactactgtgcccggagcggctggctggtgcacggggactattattttgattattggggccagggcaccacactgacagtgagcagcgaacaaaaactcatctcagaagaggatctggtgaagctgagcaaagaggccaagcagagactacagcagctcttcaaggggagccagtttgccattcgctggggctttatccctcttgtgatttacctgggatttaagaggggtgcagatcccggaatgcctgaaccaactgttttgagcctactttggggataa

SEQ ID NO: 94 - protein, 314 aa, Artificial Sequence
  amino acid sequence of scFvPDL1-myc-TOM7
MDIVMSQSPSSLAVSAGEKVTMSCKSSQSLLNSRTRKNYLAWYQQKPGQSPKLLIYWASTRESGVPDRFTGSGSGTDFTLTISSVQAEDLAVYYCQQSYDVVTFGAGTKLELKGGGGSGGGGSGGGGSQVQVQQSGAELAEPGASVKMSCKASGYIFTSYWMHWLKQRPGQGLEWIGYINPSSDYNEYSEKFMDKATLTADKASTTAYMQLISLTSEDSAVYYCARSGWLVHGDYYFDYWGQGTTLTVSSEQKLISEEDLVKLSKEAKQRLQQLFKGSQFAIRWGFIPLVIYLGFKRGADPGMPEPTVLSLLWG

SEQ ID NO: 95 - DNA, 732 bp, Artificial Sequence
  nucleotides sequence coding scFvHER2
atggaagtgcaacttgttgagagtggcggaggactggtccaaccgggcggttcacttaggctctcatgtgcagcttcagggttcacgttcacggactatacaatggactgggtgaggcaagcccctggtaagggactggagtgggttgctgacgttaaccctaattccggtgggtccatctacaaccagcgattcaagggacgatttactctttcagtcgacagaagcaaaaacaccctctacctccagatgaactccttgcgggcagaggatacagcggtctactattgcgcgagaaacttgggaccaagcttctacttcgactactgggggcaaggaacgcttgttacggtttcaagcggaggtggaggaagtggaggtggcggttccggcggtggcggttcagatatacagatgacccaatcacccagttctcttagcgcgtctgtaggcgacagggtaaccataacctgcaaggcgtcccaggacgtgtcaattggagttgcctggtatcagcaaaaacctgggaaagctccgaagctcctgatttacagcgcatcttaccgatatactggtgtcccttcaaggttcagtggcagtggatctgggacagactttacgcttactatcagcagtctgcaacctgaggatttcgcgacctactactgtcagcagtattacatctatccgtacacgttcggtcaaggtacaaaggtagaaataaaacgcact

SEQ ID NO: 96 - protein, 244 aa, Artificial Sequence
  amino acid sequence of scFvHER2
MEVQLVESGGGLVQPGGSLRLSCAASGFTFTDYTMDWVRQAPGKGLEWVADVNPNSGGSIYNQRFKGRFTLSVDRSKNTLYLQMNSLRAEDTAVYYCARNLGPSFYFDYWGQGTLVTVSSGGGGSGGGGSGGGGSDIQMTQSPSSLSASVGDRVTITCKASQDVSIGVAWYQQKPGKAPKLLIYSASYRYTGVPSRFSGSGSGTDFTLTISSLQPEDFATYYCQQYYIYPYTFGQGTKVEIKRT

SEQ ID NO: 97 - DNA, 927 bp, Artificial Sequence
  nucleotides sequence coding scFvHER2-myc-TOM7
atggaagtgcaacttgttgagagtggcggaggactggtccaaccgggcggttcacttaggctctcatgtgcagcttcagggttcacgttcacggactatacaatggactgggtgaggcaagcccctggtaagggactggagtgggttgctgacgttaaccctaattccggtgggtccatctacaaccagcgattcaagggacgatttactctttcagtcgacagaagcaaaaacaccctctacctccagatgaactccttgcgggcagaggatacagcggtctactattgcgcgagaaacttgggaccaagcttctacttcgactactgggggcaaggaacgcttgttacggtttcaagcggaggtggaggaagtggaggtggcggttccggcggtggcggttcagatatacagatgacccaatcacccagttctcttagcgcgtctgtaggcgacagggtaaccataacctgcaaggcgtcccaggacgtgtcaattggagttgcctggtatcagcaaaaacctgggaaagctccgaagctcctgatttacagcgcatcttaccgatatactggtgtcccttcaaggttcagtggcagtggatctgggacagactttacgcttactatcagcagtctgcaacctgaggatttcgcgacctactactgtcagcagtattacatctatccgtacacgttcggtcaaggtacaaaggtagaaataaaacgcactgaacaaaaactcatctcagaagaggatctggtgaagctgagcaaagaggccaagcagagactacagcagctcttcaaggggagccagtttgccattcgctggggctttatccctcttgtgatttacctgggatttaagaggggtgcagatcccggaatgcctgaaccaactgttttgagcctactttggggataa

SEQ ID NO: 98 - protein, 308 aa, Artificial Sequence
  amino acid sequence of scFvHER2-myc-TOM7
MEVQLVESGGGLVQPGGSLRLSCAASGFTFTDYTMDWVRQAPGKGLEWVADVNPNSGGSIYNQRFKGRFTLSVDRSKNTLYLQMNSLRAEDTAVYYCARNLGPSFYFDYWGQGTLVTVSSGGGGSGGGGSGGGGSDIQMTQSPSSLSASVGDRVTITCKASQDVSIGVAWYQQKPGKAPKLLIYSASYRYTGVPSRFSGSGSGTDFTLTISSLQPEDFATYYCQQYYIYPYTFGQGTKVEIKRTEQKLISEEDLVKLSKEAKQRLQQLFKGSQFAIRWGFIPLVIYLGFKRGADPGMPEPTVLSLLWG

SEQ ID NO: 99 - DNA, 726 bp, Artificial Sequence
  nucleotides sequence coding scFvMSLN
atgcaagtgcagctcgtccagtctggggctgaggtgaagaggcctggagccagtgttcaggtgtcctgccgggcctctggctacagcatcaacacctactatatgcagtgggtgcggcaggcccctggggccggcctggagtggatgggcgtcatcaatcccagcggggtgacctcctatgcccagaagttccagggccgcgtgactctcaccaatgacaccagcaccaacacagtctacatgcagctgaacagcctcacttcagctgacacagctgtgtactactgtgcccgctgggccctgtggggagactttggcatggatgtgtggggcaagggcactctggtgacagtgagcagtggagggggcggcagcggtggcggtggaagtggcggaggaggcagtgacatccagatgacccagagcccctccacactgtctgcttccatcggggacagagtcaccatcacctgccgcgccagcgagggcatctaccactggctggcctggtaccagcagaaaccaggaaaagcccccaagctgctgatttacaaggcctcctccctggcttcaggcgccccaagccgcttcagcggctccggctctggaacagacttcaccctgacaatcagcagcctgcagccagatgattttgccacctattactgccagcagtactccaactaccccctgaccttcggcgggggcaccaagttggagatcaag

SEQ ID NO: 100 - protein, 242 aa, Artificial Sequence
  amino acid sequence of scFvMSLN
MQVQLVQSGAEVKRPGASVQVSCRASGYSINTYYMQWVRQAPGAGLEWMGVINPSGVTSYAQKFQGRVTLTNDTSTNTVYMQLNSLTSADTAVYYCARWALWGDFGMDVWGKGTLVTVSSGGGGSGGGGSGGGGSDIQMTQSPSTLSASIGDRVTITCRASEGIYHWLAWYQQKPGKAPKLLIYKASSLASGAPSRFSGSGSGTDFTLTISSLQPDDFATYYCQQYSNYPLTFGGGTKLEIK

SEQ ID NO: 101 - DNA, 921 bp, Artificial Sequence
  nucleotides sequence coding scFvMSLN-myc-TOM7
atgcaagtgcagctcgtccagtctggggctgaggtgaagaggcctggagccagtgttcaggtgtcctgccgggcctctggctacagcatcaacacctactatatgcagtgggtgcggcaggcccctggggccggcctggagtggatgggcgtcatcaatcccagcggggtgacctcctatgcccagaagttccagggccgcgtgactctcaccaatgacaccagcaccaacacagtctacatgcagctgaacagcctcacttcagctgacacagctgtgtactactgtgcccgctgggccctgtggggagactttggcatggatgtgtggggcaagggcactctggtgacagtgagcagtggagggggcggcagcggtggcggtggaagtggcggaggaggcagtgacatccagatgacccagagcccctccacactgtctgcttccatcggggacagagtcaccatcacctgccgcgccagcgagggcatctaccactggctggcctggtaccagcagaaaccaggaaaagcccccaagctgctgatttacaaggcctcctccctggcttcaggcgccccaagccgcttcagcggctccggctctggaacagacttcaccctgacaatcagcagcctgcagccagatgattttgccacctattactgccagcagtactccaactaccccctgaccttcggcgggggcaccaagttggagatcaaggaacaaaaactcatctcagaagaggatctggtgaagctgagcaaagaggccaagcagagactacagcagctcttcaaggggagccagtttgccattcgctggggctttatccctcttgtgatttacctgggatttaagaggggtgcagatcccggaatgcctgaaccaactgttttgagcctactttggggataa

SEQ ID NO: 102 - protein, 306 aa, Artificial Sequence
  amino acid sequence of scFvMSLN-myc-TOM7
MQVQLVQSGAEVKRPGASVQVSCRASGYSINTYYMQWVRQAPGAGLEWMGVINPSGVTSYAQKFQGRVTLTNDTSTNTVYMQLNSLTSADTAVYYCARWALWGDFGMDVWGKGTLVTVSSGGGGSGGGGSGGGGSDIQMTQSPSTLSASIGDRVTITCRASEGIYHWLAWYQQKPGKAPKLLIYKASSLASGAPSRFSGSGSGTDFTLTISSLQPDDFATYYCQQYSNYPLTFGGGTKLEIKEQKLISEEDLVKLSKEAKQRLQQLFKGSQFAIRWGFIPLVIYLGFKRGADPGMPEPTVLSLLWG